European Patent Specification EP 3 729 081 B1, published February 19, 2025. Title: CAR-T cell assay for specificity test of novel antigen binding moieties. Applicant: F.Hoffmann-La Roche Ltd. The sequence listing filed with the application follows.

SEQUENCE LISTING (93 sequences)

SEQ ID NO: 1 - protein, 5 aa, Artificial sequence
  Anti-CD20 ( GA101)  CDR H1 Kabat
YSWIN

SEQ ID NO: 2 - protein, 17 aa, Artificial sequence
  Anti-CD20 ( GA101)  CDR H2 Kabat
RIFPGDGDTDYNGKFKG

SEQ ID NO: 3 - protein, 10 aa, Artificial sequence
  Anti-CD20 ( GA101)  CDR H3 Kabat
NVFDGYWLVY

SEQ ID NO: 4 - protein, 16 aa, Artificial sequence
  Anti-CD20 ( GA101)  CDR L1 Kabat
RSSKSLLHSNGITYLY

SEQ ID NO: 5 - protein, 7 aa, Artificial sequence
  Anti-CD20 ( GA101)  CDR L2 Kabat
QMSNLVS

SEQ ID NO: 6 - protein, 9 aa, Artificial sequence
  Anti-CD20 ( GA101)  CDR L3 Kabat
AQNLELPYT

SEQ ID NO: 7 - protein, 407 aa, Artificial sequence
  Anti-CD20-(GA101)-Fab heavy chain-CD28ATD-CD28CSD-CD3zSSD fusion pETR 17097
QVQLVQSGAEVKKPGSSVKVSCKASGYAFSYSWINWVRQAPGQGLEWMGRIFPGDGDTDYNGKFKGRVTITADKSTSTAYMELSSLRSEDTAVYYCARNVFDGYWLVYWGQGTLVTVSSASTKGPSVFPLAPSSKSTSGGTAALGCLVKDYFPEPVTVSWNSGALTSGVHTFPAVLQSSGLYSLSSVVTVPSSSLGTQTYICNVNHKPSNTKVDKKVEPKSCGGGGSFWVLVVVGGVLACYSLLVTVAFIIFWVRSKRSRLLHSDYMNMTPRRPGPTRKHYQPYAPPRDFAAYRSRVKFSRSADAPAYQQGQNQLYNELNLGRREEYDVLDKRRGRDPEMGGKPRRKNPQEGLYNELQKDKMAEAYSEIGMKGERRRGKGHDGLYQGLSTATKDTYDALHMQALPPR

SEQ ID NO: 8 - protein, 222 aa, Artificial sequence
  Anti-CD20-(GA101)-Fab heavy chain
QVQLVQSGAEVKKPGSSVKVSCKASGYAFSYSWINWVRQAPGQGLEWMGRIFPGDGDTDYNGKFKGRVTITADKSTSTAYMELSSLRSEDTAVYYCARNVFDGYWLVYWGQGTLVTVSSASTKGPSVFPLAPSSKSTSGGTAALGCLVKDYFPEPVTVSWNSGALTSGVHTFPAVLQSSGLYSLSSVVTVPSSSLGTQTYICNVNHKPSNTKVDKKVEPKSC

SEQ ID NO: 9 - protein, 219 aa, Artificial sequence
  Anti-CD20-(GA101)-Fab light chain
DIVMTQTPLSLPVTPGEPASISCRSSKSLLHSNGITYLYWYLQKPGQSPQLLIYQMSNLVSGVPDRFSGSGSGTDFTLKISRVEAEDVGVYYCAQNLELPYTFGGGTKVEIKRTVAAPSVFIFPPSDEQLKSGTASVVCLLNNFYPREAKVQWKVDNALQSGNSQESVTEQDSKDSTYSLSSTLTLSKADYEKHKVYACEVTHQGLSSPVTKSFNRGEC

SEQ ID NO: 10 - protein, 112 aa, Artificial sequence
  Anti-CD20-(GA101) VL
DIVMTQTPLSLPVTPGEPASISCRSSKSLLHSNGITYLYWYLQKPGQSPQLLIYQMSNLVSGVPDRFSGSGSGTDFTLKISRVEAEDVGVYYCAQNLELPYTFGGGTKVEIK

SEQ ID NO: 11 - protein, 107 aa, Artificial sequence [sequence omitted]

SEQ ID NO: 12 - protein, 119 aa, Artificial sequence
  Anti-CD20-(GA101) VH
QVQLVQSGAEVKKPGSSVKVSCKASGYAFSYSWINWVRQAPGQGLEWMGRIFPGDGDTDYNGKFKGRVTITADKSTSTAYMELSSLRSEDTAVYYCARNVFDGYWLVYWGQGTLVTVSS

SEQ ID NO: 13 - protein, 103 aa, Artificial sequence
  CH1
ASTKGPSVFPLAPSSKSTSGGTAALGCLVKDYFPEPVTVSWNSGALTSGVHTFPAVLQSSGLYSLSSVVTVPSSSLGTQTYICNVNHKPSNTKVDKKVEPKSC

SEQ ID NO: 14 - protein, 27 aa, Artificial sequence
  CD28ATD
FWVLVVVGGVLACYSLLVTVAFIIFWV

SEQ ID NO: 15 - protein, 41 aa, Artificial sequence
  CD28CSD
RSKRSRLLHSDYMNMTPRRPGPTRKHYQPYAPPRDFAAYRS

SEQ ID NO: 16 - protein, 112 aa, Artificial sequence
  CD3zSSD
RVKFSRSADAPAYQQGQNQLYNELNLGRREEYDVLDKRRGRDPEMGGKPRRKNPQEGLYNELQKDKMAEAYSEIGMKGERRRGKGHDGLYQGLSTATKDTYDALHMQALPPR

SEQ ID NO: 17 - protein, 180 aa, Artificial sequence
  CD28ATD-CD28CSD-CD3zSSD
FWVLVVVGGVLACYSLLVTVAFIIFWVRSKRSRLLHSDYMNMTPRRPGPTRKHYQPYAPPRDFAAYRSRVKFSRSADAPAYQQGQNQLYNELNLGRREEYDVLDKRRGRDPEMGGKPRRKNPQEGLYNELQKDKMAEAYSEIGMKGERRRGKGHDGLYQGLSTATKDTYDALHMQALPPR

SEQ ID NO: 18 - protein, 238 aa, Artificial sequence
  eGFP
VSKGEELFTGVVPILVELDGDVNGHKFSVSGEGEGDATYGKLTLKFICTTGKLPVPWPTLVTTLTYGVQCFSRYPDHMKQHDFFKSAMPEGYVQERTIFFKDDGNYKTRAEVKFEGDTLVNRIELKGIDFKEDGNILGHKLEYNYNSHNVYIMADKQKNGIKVNFKIRHNIEDGSVQLADHYQQNTPIGDGPVLLPDNHYLSTQSALSKDPNEKRDHMVLLEFVTAAGITLGMDELYK

SEQ ID NO: 19 - protein, 20 aa, Artificial sequence
  (G4S)4 linker
GGGGSGGGGSGGGGSGGGGS

SEQ ID NO: 20 - protein, 5 aa, Artificial sequence
  G4S linker
GGGGS

SEQ ID NO: 21 - protein, 19 aa, Artificial sequence
  T2A linker
GEGRGSLLTCGDVEENPGP

SEQ ID NO: 22 - DNA, 2659 bp, Artificial sequence
  Anti-CD20-(GA101)-Fab-CD28ATD-CD28CSD-CD3zSSD pETR17097
atgggatggagctgtatcatcctcttcttggtagcaacagctaccggtgtgcattccgatatcgtgatgacccagactccactctccctgcccgtcacccctggagagcccgccagcattagctgcaggtctagcaagagcctcttgcacagcaatggcatcacttatttgtattggtacctgcaaaagccagggcagtctccacagctcctgatttatcaaatgtccaaccttgtctctggcgtccctgaccggttctccggatccgggtcaggcactgatttcacactgaaaatcagcagggtggaggctgaggatgttggagtttattactgcgctcagaatctagaacttccttacaccttcggcggagggaccaaggtggagatcaaaccgtacggtggctgcaccatctgtcttcatcttcccgccatctgatgagcagttgaaatctggaactgcctctgttgtgtgcctgctgaataacttctatcccagagaggccaaagtacagtggaaggtggataacgccctccaatcgggtaactcccaggagagtgtcacagagcaggacagcaaggacagcacctacagcctcagcagcaccctgacgctgagcaaagcagactacgagaaacacaaagtctacgcctgcgaagtcacccatcagggcctgagctcgcccgtcacaaagagcttcaacaggggagagtgttagaatagaattccccgaagtaacttagaagctgtaaatcaacgatcaatagcaggtgtggcacaccagtcataccttgatcaagcacttctgtttccccggactgagtatcaataggctgctcgcgcggctgaaggagaaaacgttcgttacccgaccaactacttcgagaagcttagtaccaccatgaacgaggcagggtgtttcgctcagcacaaccccagtgtagatcaggctgatgagtcactgcaacccccatgggcgaccatggcagtggctgcgttggcggcctgcccatggagaaatccatgggacgctctaattctgacatggtgtgaagtgcctattgagctaactggtagtcctccggcccctgattgcggctaatcctaactgcggagcacatgctcacaaaccagtgggtggtgtgtcgtaacgggcaactctgcagcggaaccgactactttgggtgtccgtgtttccttttattcctatattggctgcttatggtgacaatcaaaaagttgttaccatatagctattggattggccatccggtgtgcaacagggcaactgtttacctatttattggttttgtaccattatcactgaagtctgtgatcactctcaaattcattttgaccctcaacacaatcaaacgccaccatgggatggagctgtatcatcctcttcttggtagcaacagctaccggtgtgcactcccaggtgcaattggtgcagtctggcgctgaagttaagaagcctgggagttcagtgaaggtctcctgcaaggcttcgggatacgccttcagctattcttggatcaattgggtgcggcaggcgcctggacaagggctcgagtggatgggacggatctttcccggcgatggggatactgactacaatgggaaattcaagggcagagtcacaattaccgccgacaaatccactagcacagcctatatggagctgagcagcctgagatctgaggacacggccgtgtattactgtgcaagaaatgtctttgatggttactggcttgtttactggggccagggaaccctggtcaccgtctccagcgctagcaccaagggcccctccgtgttccccctggcccccagcagcaagagcaccagcggcggcacagccgctctgggctgcctggtcaaggactacttccccgagcccgtgaccgtgtcctggaacagcggagccctgacctccggcgtgcacaccttccccgccgtgctgcagagttctggcctgtatagcctgagcagcgtggtcaccgtgccttctagcagcctgggcacccagacctacatctgcaacgtgaaccacaagcccagcaacaccaaggtggacaagaaggtggagcccaagagctgcggagggggcggatccttctgggtgctggtggtggtgggcggcgtgctggcctgctacagcctgctggtgaccgtggccttcatcatcttctgggtgaggagcaagaggagcaggctgctgcacagcgactacatgaacatgacccccaggaggcccggccccaccaggaagcactaccagccctacgccccccccagggacttcgccgcctacaggagcagggtgaagttcagcaggagcgccgacgcccccgcctaccagcagggccagaaccagctgtataacgagctgaacctgggcaggagggaggagtacgacgtgctggacaagaggaggggcagggaccccgagatgggcggcaagcccaggaggaagaacccccaggagggcctgtataacgagctgcagaaggacaagatggccgaggcctacagcgagatcggcatgaagggcgagaggaggaggggcaagggccacgacggcctgtaccagggcctgagcaccgccaccaaggacacctacgacgccctgcacatgcaggccctgccccccagg

SEQ ID NO: 23 - DNA, 336 bp, Artificial sequence
  Anti-CD20-(GA101)-Fab-VL
gatatcgtgatgacccagactccactctccctgcccgtcacccctggagagcccgccagcattagctgcaggtctagcaagagcctcttgcacagcaatggcatcacttatttgtattggtacctgcaaaagccagggcagtctccacagctcctgatttatcaaatgtccaaccttgtctctggcgtccctgaccggttctccggatccgggtcaggcactgatttcacactgaaaatcagcagggtggaggctgaggatgttggagtttattactgcgctcagaatctagaacttccttacaccttcggcggagggaccaaggtggagatcaaa

SEQ ID NO: 24 - DNA, 324 bp, Artificial sequence
  Fab CL
cgtacggtggctgcaccatctgtcttcatcttcccgccatctgatgagcagttgaaatctggaactgcctctgttgtgtgcctgctgaataacttctatcccagagaggccaaagtacagtggaaggtggataacgccctccaatcgggtaactcccaggagagtgtcacagagcaggacagcaaggacagcacctacagcctcagcagcaccctgacgctgagcaaagcagactacgagaaacacaaagtctacgcctgcgaagtcacccatcagggcctgagctcgcccgtcacaaagagcttcaacaggggagagtgttag

SEQ ID NO: 25 - DNA, 357 bp, Artificial sequence
  Anti-CD20-(GA101)-Fab-VH
caggtgcaattggtgcagtctggcgctgaagttaagaagcctgggagttcagtgaaggtctcctgcaaggcttcgggatacgccttcagctattcttggatcaattgggtgcggcaggcgcctggacaagggctcgagtggatgggacggatctttcccggcgatggggatactgactacaatgggaaattcaagggcagagtcacaattaccgccgacaaatccactagcacagcctatatggagctgagcagcctgagatctgaggacacggccgtgtattactgtgcaagaaatgtctttgatggttactggcttgtttactggggccagggaaccctggtcaccgtctccagc

SEQ ID NO: 26 - DNA, 309 bp, Artificial sequence
  Fab CH1
gctagcaccaagggcccctccgtgttccccctggcccccagcagcaagagcaccagcggcggcacagccgctctgggctgcctggtcaaggactacttccccgagcccgtgaccgtgtcctggaacagcggagccctgacctccggcgtgcacaccttccccgccgtgctgcagagttctggcctgtatagcctgagcagcgtggtcaccgtgccttctagcagcctgggcacccagacctacatctgcaacgtgaaccacaagcccagcaacaccaaggtggacaagaaggtggagcccaagagctgc

SEQ ID NO: 27 - DNA, 647 bp, Artificial sequence
  IRES EV71 internal ribosomal entry side
cccgaagtaacttagaagctgtaaatcaacgatcaatagcaggtgtggcacaccagtcataccttgatcaagcacttctgtttccccggactgagtatcaataggctgctcgcgcggctgaaggagaaaacgttcgttacccgaccaactacttcgagaagcttagtaccaccatgaacgaggcagggtgtttcgctcagcacaaccccagtgtagatcaggctgatgagtcactgcaacccccatgggcgaccatggcagtggctgcgttggcggcctgcccatggagaaatccatgggacgctctaattctgacatggtgtgaagtgcctattgagctaactggtagtcctccggcccctgattgcggctaatcctaactgcggagcacatgctcacaaaccagtgggtggtgtgtcgtaacgggcaactctgcagcggaaccgactactttgggtgtccgtgtttccttttattcctatattggctgcttatggtgacaatcaaaaagttgttaccatatagctattggattggccatccggtgtgcaacagggcaactgtttacctatttattggttttgtaccattatcactgaagtctgtgatcactctcaaattcattttgaccctcaacacaatcaaac

SEQ ID NO: 28 - DNA, 15 bp, Artificial sequence
  G4S linker
ggagggggcggatcc

SEQ ID NO: 29 - DNA, 81 bp, Artificial sequence
  CD28ATD
ttttgggtgctggtggtggttggtggagtcctggcttgctatagcttgctagtaacagtggcctttattattttctgggtg

SEQ ID NO: 30 - DNA, 123 bp, Artificial sequence
  CD28CSD
aggagtaagaggagcaggctcctgcacagtgactacatgaacatgactccccgccgccccgggcccacccgcaagcattaccagccctatgccccaccacgcgacttcgcagcctatcgctcc

SEQ ID NO: 31 - DNA, 336 bp, Artificial sequence
  CD3zSSD
agagtgaagttcagcaggagcgcagacgcccccgcgtaccagcagggccagaaccagctctataacgagctcaatctaggacgaagagaggagtacgatgttttggacaagagacgtggccgggaccctgagatggggggaaagccgagaaggaagaaccctcaggaaggcctgtacaatgaactgcagaaagataagatggcggaggcctacagtgagattgggatgaaaggcgagcgccggaggggcaaggggcacgatggcctttaccagggtctcagtacagccaccaaggacacctacgacgcccttcacatgcaggccctgccccctcgc

SEQ ID NO: 32 - DNA, 540 bp, Artificial sequence
  CD28ATD-CD28CSD-CD3zSSD
ttctgggtgctggtggtggtgggcggcgtgctggcctgctacagcctgctggtgaccgtggccttcatcatcttctgggtgaggagcaagaggagcaggctgctgcacagcgactacatgaacatgacccccaggaggcccggccccaccaggaagcactaccagccctacgccccccccagggacttcgccgcctacaggagcagggtgaagttcagcaggagcgccgacgcccccgcctaccagcagggccagaaccagctgtataacgagctgaacctgggcaggagggaggagtacgacgtgctggacaagaggaggggcagggaccccgagatgggcggcaagcccaggaggaagaacccccaggagggcctgtataacgagctgcagaaggacaagatggccgaggcctacagcgagatcggcatgaagggcgagaggaggaggggcaagggccacgacggcctgtaccagggcctgagcaccgccaccaaggacacctacgacgccctgcacatgcaggccctgccccccagg

SEQ ID NO: 33 - DNA, 63 bp, Artificial sequence
  T2A linker
tccggagagggcagaggaagtcttctaacatgcggtgacgtggaggagaatcccggccctagg

SEQ ID NO: 34 - DNA, 717 bp, Artificial sequence
  eGFP
gtgagcaagggcgaggagctgttcaccggggtggtgcccatcctggtcgagctggacggcgacgtaaacggccacaagttcagcgtgtccggcgagggcgagggcgatgccacctacggcaagctgaccctgaagttcatctgcaccaccggcaagctgcccgtgccctggcccaccctcgtgaccaccctgacctacggcgtgcagtgcttcagccgctaccccgaccacatgaagcagcacgacttcttcaagtccgccatgcccgaaggctacgtccaggagcgcaccatcttcttcaaggacgacggcaactacaagacccgcgccgaggtgaagttcgagggcgacaccctggtgaaccgcatcgagctgaagggcatcgacttcaaggaggacggcaacatcctggggcacaagctggagtacaactacaacagccacaacgtctatatcatggccgacaagcagaagaacggcatcaaggtgaacttcaagatccgccacaacatcgaggacggcagcgtgcagctcgccgaccactaccagcagaacacccccatcggcgacggccccgtgctgctgcccgacaaccactacctgagcacccagtccgccctgagcaaagaccccaacgagaagcgcgatcacatggtcctgctggagttcgtgaccgccgccgggatcactctcggcatggacgagctgtacaagtga

SEQ ID NO: 35 - DNA, 3438 bp, Artificial sequence
  Anti-CD20-(GA101)-Fab-CD28ATD-CD28CSD-CD3zSSD-eGFP pETR17097
atgggatggagctgtatcatcctcttcttggtagcaacagctaccggtgtgcattccgatatcgtgatgacccagactccactctccctgcccgtcacccctggagagcccgccagcattagctgcaggtctagcaagagcctcttgcacagcaatggcatcacttatttgtattggtacctgcaaaagccagggcagtctccacagctcctgatttatcaaatgtccaaccttgtctctggcgtccctgaccggttctccggatccgggtcaggcactgatttcacactgaaaatcagcagggtggaggctgaggatgttggagtttattactgcgctcagaatctagaacttccttacaccttcggcggagggaccaaggtggagatcaaacgtacggtggctgcaccatctgtcttcatcttcccgccatctgatgagcagttgaaatctggaactgcctctgttgtgtgcctgctgaataacttctatcccagagaggccaaagtacagtggaaggtggataacgccctccaatcgggtaactcccaggagagtgtcacagagcaggacagcaaggacagcacctacagcctcagcagcaccctgacgctgagcaaagcagactacgagaaacacaaagtctacgcctgcgaagtcacccatcagggcctgagctcgcccgtcacaaagagcttcaacaggggagagtgttagaatagaattccccgaagtaacttagaagctgtaaatcaacgatcaatagcaggtgtggcacaccagtcataccttgatcaagcacttctgtttccccggactgagtatcaataggctgctcgcgcggctgaaggagaaaacgttcgttacccgaccaactacttcgagaagcttagtaccaccatgaacgaggcagggtgtttcgctcagcacaaccccagtgtagatcaggctgatgagtcactgcaacccccatgggcgaccatggcagtggctgcgttggcggcctgcccatggagaaatccatgggacgctctaattctgacatggtgtgaagtgcctattgagctaactggtagtcctccggcccctgattgcggctaatcctaactgcggagcacatgctcacaaaccagtgggtggtgtgtcgtaacgggcaactctgcagcggaaccgactactttgggtgtccgtgtttccttttattcctatattggctgcttatggtgacaatcaaaaagttgttaccatatagctattggattggccatccggtgtgcaacagggcaactgtttacctatttattggttttgtaccattatcactgaagtctgtgatcactctcaaattcattttgaccctcaacacaatcaaacgccaccatgggatggagctgtatcatcctcttcttggtagcaacagctaccggtgtgcactcccaggtgcaattggtgcagtctggcgctgaagttaagaagcctgggagttcagtgaaggtctcctgcaaggcttcgggatacgccttcagctattcttggatcaattgggtgcggcaggcgcctggacaagggctcgagtggatgggacggatctttcccggcgatggggatactgactacaatgggaaattcaagggcagagtcacaattaccgccgacaaatccactagcacagcctatatggagctgagcagcctgagatctgaggacacggccgtgtattactgtgcaagaaatgtctttgatggttactggcttgtttactggggccagggaaccctggtcaccgtctccagcgctagcaccaagggcccctccgtgttccccctggcccccagcagcaagagcaccagcggcggcacagccgctctgggctgcctggtcaaggactacttccccgagcccgtgaccgtgtcctggaacagcggagccctgacctccggcgtgcacaccttccccgccgtgctgcagagttctggcctgtatagcctgagcagcgtggtcaccgtgccttctagcagcctgggcacccagacctacatctgcaacgtgaaccacaagcccagcaacaccaaggtggacaagaaggtggagcccaagagctgcggagggggcggatccttctgggtgctggtggtggtgggcggcgtgctggcctgctacagcctgctggtgaccgtggccttcatcatcttctgggtgaggagcaagaggagcaggctgctgcacagcgactacatgaacatgacccccaggaggcccggccccaccaggaagcactaccagccctacgccccccccagggacttcgccgcctacaggagcagggtgaagttcagcaggagcgccgacgcccccgcctaccagcagggccagaaccagctgtataacgagctgaacctgggcaggagggaggagtacgacgtgctggacaagaggaggggcagggaccccgagatgggcggcaagcccaggaggaagaacccccaggagggcctgtataacgagctgcagaaggacaagatggccgaggcctacagcgagatcggcatgaagggcgagaggaggaggggcaagggccacgacggcctgtaccagggcctgagcaccgccaccaaggacacctacgacgccctgcacatgcaggccctgccccccaggtccggagagggcagaggaagtcttctaacatgcggtgacgtggaggagaatcccggccctagggtgagcaagggcgaggagctgttcaccggggtggtgcccatcctggtcgagctggacggcgacgtaaacggccacaagttcagcgtgtccggcgagggcgagggcgatgccacctacggcaagctgaccctgaagttcatctgcaccaccggcaagctgcccgtgccctggcccaccctcgtgaccaccctgacctacggcgtgcagtgcttcagccgctaccccgaccacatgaagcagcacgacttcttcaagtccgccatgcccgaaggctacgtccaggagcgcaccatcttcttcaaggacgacggcaactacaagacccgcgccgaggtgaagttcgagggcgacaccctggtgaaccgcatcgagctgaagggcatcgacttcaaggaggacggcaacatcctggggcacaagctggagtacaactacaacagccacaacgtctatatcatggccgacaagcagaagaacggcatcaaggtgaacttcaagatccgccacaacatcgaggacggcagcgtgcagctcgccgaccactaccagcagaacacccccatcggcgacggccccgtgctgctgcccgacaaccactacctgagcacccagtccgccctgagcaaagaccccaacgagaagcgcgatcacatggtcctgctggagttcgtgaccgccgccgggatcactctcggcatggacgagctgtacaagtga

SEQ ID NO: 36 - protein, 411 aa, Artificial sequence
  Anti-CD20-(GA101)-crossFab VH-CL light chain-ATD-CD28ATD-CD28CSD-CD3zSSD fusion pETR17098
QVQLVQSGAEVKKPGSSVKVSCKASGYAFSYSWINWVRQAPGQGLEWMGRIFPGDGDTDYNGKFKGRVTITADKSTSTAYMELSSLRSEDTAVYYCARNVFDGYWLVYWGQGTLVTVSSASVAAPSVFIFPPSDEQLKSGTASVVCLLNNFYPREAKVQWKVDNALQSGNSQESVTEQDSKDSTYSLSSTLTLSKADYEKHKVYACEVTHQGLSSPVTKSFNRGECGGGGSFWVLVVVGGVLACYSLLVTVAFIIFWVRSKRSRLLHSDYMNMTPRRPGPTRKHYQPYAPPRDFAAYRSRVKFSRSADAPAYQQGQNQLYNELNLGRREEYDVLDKRRGRDPEMGGKPRRKNPQEGLYNELQKDKMAEAYSEIGMKGERRRGKGHDGLYQGLSTATKDTYDALHMQALPPR

SEQ ID NO: 37 - protein, 226 aa, Artificial sequence
  Anti-CD20-(GA101)-crossFab VH-CL light chain pETR17098
QVQLVQSGAEVKKPGSSVKVSCKASGYAFSYSWINWVRQAPGQGLEWMGRIFPGDGDTDYNGKFKGRVTITADKSTSTAYMELSSLRSEDTAVYYCARNVFDGYWLVYWGQGTLVTVSSASVAAPSVFIFPPSDEQLKSGTASVVCLLNNFYPREAKVQWKVDNALQSGNSQESVTEQDSKDSTYSLSSTLTLSKADYEKHKVYACEVTHQGLSSPVTKSFNRGEC

SEQ ID NO: 38 - protein, 217 aa, Artificial sequence
  Anti-CD20-(GA101)-crossFab VL-CH1 heavy chain-pETR17098
DIVMTQTPLSLPVTPGEPASISCRSSKSLLHSNGITYLYWYLQKPGQSPQLLIYQMSNLVSGVPDRFSGSGSGTDFTLKISRVEAEDVGVYYCAQNLELPYTFGGGTKVEIKSSASTKGPSVFPLAPSSKSTSGGTAALGCLVKDYFPEPVTVSWNSGALTSGVHTFPAVLQSSGLYSLSSVVTVPSSSLGTQTYICNVNHKPSNTKVDKKVEPKSC

SEQ ID NO: 39 - protein, 107 aa, Artificial sequence
  crossFab CL
ASVAAPSVFIFPPSDEQLKSGTASVVCLLNNFYPREAKVQWKVDNALQSGNSQESVTEQDSKDSTYSLSSTLTLSKADYEKHKVYACEVTHQGLSSPVTKSFNRGEC

SEQ ID NO: 40 - protein, 105 aa, Artificial sequence
  crossFab CH1
SSASTKGPSVFPLAPSSKSTSGGTAALGCLVKDYFPEPVTVSWNSGALTSGVHTFPAVLQSSGLYSLSSVVTVPSSSLGTQTYICNVNHKPSNTKVDKKVEPKSC

SEQ ID NO: 41 - protein, 402 aa, Artificial sequence
  Anti-CD20-(GA101)-crossFab VL-CH1 heavy-chain-ATD-CD28ATD-CD28CSD-CD3zSSD fusion
DIVMTQTPLSLPVTPGEPASISCRSSKSLLHSNGITYLYWYLQKPGQSPQLLIYQMSNLVSGVPDRFSGSGSGTDFTLKISRVEAEDVGVYYCAQNLELPYTFGGGTKVEIKSSASTKGPSVFPLAPSSKSTSGGTAALGCLVKDYFPEPVTVSWNSGALTSGVHTFPAVLQSSGLYSLSSVVTVPSSSLGTQTYICNVNHKPSNTKVDKKVEPKSCGGGGSFWVLVVVGGVLACYSLLVTVAFIIFWVRSKRSRLLHSDYMNMTPRRPGPTRKHYQPYAPPRDFAAYRSRVKFSRSADAPAYQQGQNQLYNELNLGRREEYDVLDKRRGRDPEMGGKPRRKNPQEGLYNELQKDKMAEAYSEIGMKGERRRGKGHDGLYQGLSTATKDTYDALHMQALPPR

SEQ ID NO: 42 - protein, 217 aa, Artificial sequence; identical to SEQ ID NO: 38
  Anti-CD20-(GA101)-crossFab VL-CH1 heavy chain

SEQ ID NO: 43 - protein, 226 aa, Artificial sequence; identical to SEQ ID NO: 37
  Anti-CD20-(GA101)-crossFab VH-CL light chain

SEQ ID NO: 44 - protein, 107 aa, Artificial sequence; identical to SEQ ID NO: 39
  crossFab CL

SEQ ID NO: 45 - protein, 105 aa, Artificial sequence; identical to SEQ ID NO: 40
  crossFab CH1

SEQ ID NO: 46 - DNA, 2664 bp, Artificial sequence
  Anti-CD20-(GA101)-crossFabVH-CL CD28ATD-CD28CSD-CD3zSSD pETR17098
atgggatggagctgtatcatcctcttcttggtagcaacagctaccggtgtgcattcccaggtgcaattggtgcagtctggcgctgaagttaagaagcctgggagttcagtgaaggtctcctgcaaggcttccggatacgccttcagctattcttggatcaattgggtgcggcaggcgcctggacaagggctcgagtggatgggacggatctttcccggcgatggggatactgactacaatgggaaattcaagggcagagtcacaattaccgccgacaaatccactagcacagcctatatggagctgagcagcctgagatctgaggacacggccgtgtattactgtgcaagaaatgtctttgatggttactggcttgtttactggggccagggaaccctggtcaccgtctcctcagctagcgtggccgctccctccgtgttcatcttcccaccttccgacgagcagctgaagtccggcaccgcttctgtcgtgtgcctgctgaacaacttctacccccgcgaggccaaggtgcagtggaaggtggacaacgccctgcagtccggcaacagccaggaatccgtgaccgagcaggactccaaggacagcacctactccctgtcctccaccctgaccctgtccaaggccgactacgagaagcacaaggtgtacgcctgcgaagtgacccaccagggcctgtctagccccgtgaccaagtctttcaaccggggcgagtgctgataaggaattccccgaagtaacttagaagctgtaaatcaacgatcaatagcaggtgtggcacaccagtcataccttgatcaagcacttctgtttccccggactgagtatcaataggctgctcgcgcggctgaaggagaaaacgttcgttacccgaccaactacttcgagaagcttagtaccaccatgaacgaggcagggtgtttcgctcagcacaaccccagtgtagatcaggctgatgagtcactgcaacccccatgggcgaccatggcagtggctgcgttggcggcctgcccatggagaaatccatgggacgctctaattctgacatggtgtgaagtgcctattgagctaactggtagtcctccggcccctgattgcggctaatcctaactgcggagcacatgctcacaaaccagtgggtggtgtgtcgtaacgggcaactctgcagcggaaccgactactttgggtgtccgtgtttccttttattcctatattggctgcttatggtgacaatcaaaaagttgttaccatatagctattggattggccatccggtgtgcaacagggcaactgtttacctatttattggttttgtaccattatcactgaagtctgtgatcactctcaaattcattttgaccctcaacacaatcaaacgccaccatgggatggagctgtatcatcctcttcttggtagcaacagctaccggtgtgcactccgacatcgtgatgacccagactccactctccctgcccgtcacccctggagagcccgccagcattagctgcaggtctagcaagagcctcttgcacagcaatggcatcacttatttgtattggtacctgcaaaagccagggcagtctccacagctcctgatttatcaaatgtccaaccttgtctctggcgtccctgatcggttctccggttccgggtcaggcactgatttcacactgaaaatcagcagggtggaggctgaggatgttggagtttattactgcgctcagaatctagaacttccttacaccttcggcggagggaccaaggtggagatcaaatccagcgctagcaccaagggcccctccgtgttccccctggcccccagcagcaagagcaccagcggcggcacagccgctctgggctgcctggtcaaggactacttccccgagcccgtgaccgtgtcctggaacagcggagccctgacctccggcgtgcacaccttccccgccgtgctgcagagttctggcctgtatagcctgagcagcgtggtcaccgtgccttctagcagcctgggcacccagacctacatctgcaacgtgaaccacaagcccagcaacaccaaggtggacaagaaggtggagcccaagagctgcggagggggcggatccttctgggtgctggtggtggtgggcggcgtgctggcctgctacagcctgctggtgaccgtggccttcatcatcttctgggtgaggagcaagaggagcaggctgctgcacagcgactacatgaacatgacccccaggaggcccggccccaccaggaagcactaccagccctacgccccccccagggacttcgccgcctacaggagcagggtgaagttcagcaggagcgccgacgcccccgcctaccagcagggccagaaccagctgtataacgagctgaacctgggcaggagggaggagtacgacgtgctggacaagaggaggggcagggaccccgagatgggcggcaagcccaggaggaagaacccccaggagggcctgtataacgagctgcagaaggacaagatggccgaggcctacagcgagatcggcatgaagggcgagaggaggaggggcaagggccacgacggcctgtaccagggcctgagcaccgccaccaaggacacctacgacgccctgcacatgcaggccctgccccccagg

SEQ ID NO: 47 - DNA, 324 bp, Artificial sequence
  crossFab CL
gctagcgtggccgctccctccgtgttcatcttcccaccttccgacgagcagctgaagtccggcaccgcttctgtcgtgtgcctgctgaacaacttctacccccgcgaggccaaggtgcagtggaaggtggacaacgccctgcagtccggcaacagccaggaatccgtgaccgagcaggactccaaggacagcacctactccctgtcctccaccctgaccctgtccaaggccgactacgagaagcacaaggtgtacgcctgcgaagtgacccaccagggcctgtctagccccgtgaccaagtctttcaaccggggcgagtgctga

SEQ ID NO: 48 - DNA, 315 bp, Artificial sequence
  crossFab CH1
tccagcgctagcaccaagggcccctccgtgttccccctggcccccagcagcaagagcaccagcggcggcacagccgctctgggctgcctggtcaaggactacttccccgagcccgtgaccgtgtcctggaacagcggagccctgacctccggcgtgcacaccttccccgccgtgctgcagagttctggcctgtatagcctgagcagcgtggtcaccgtgccttctagcagcctgggcacccagacctacatctgcaacgtgaaccacaagcccagcaacaccaaggtggacaagaaggtggagcccaagagctgc

SEQ ID NO: 49 - DNA, 3444 bp, Artificial sequence
  Anti-CD20-(GA101)-crossFabVH-CL CD28ATD-CD28CSD-CD3zSSD-eGFP pETR17098
atgggatggagctgtatcatcctcttcttggtagcaacagctaccggtgtgcattcccaggtgcaattggtgcagtctggcgctgaagttaagaagcctgggagttcagtgaaggtctcctgcaaggcttccggatacgccttcagctattcttggatcaattgggtgcggcaggcgcctggacaagggctcgagtggatgggacggatctttcccggcgatggggatactgactacaatgggaaattcaagggcagagtcacaattaccgccgacaaatccactagcacagcctatatggagctgagcagcctgagatctgaggacacggccgtgtattactgtgcaagaaatgtctttgatggttactggcttgtttactggggccagggaaccctggtcaccgtctcctcagctagcgtggccgctccctccgtgttcatcttcccaccttccgacgagcagctgaagtccggcaccgcttctgtcgtgtgcctgctgaacaacttctacccccgcgaggccaaggtgcagtggaaggtggacaacgccctgcagtccggcaacagccaggaatccgtgaccgagcaggactccaaggacagcacctactccctgtcctccaccctgaccctgtccaaggccgactacgagaagcacaaggtgtacgcctgcgaagtgacccaccagggcctgtctagccccgtgaccaagtctttcaaccggggcgagtgctgataaggaattccccgaagtaacttagaagctgtaaatcaacgatcaatagcaggtgtggcacaccagtcataccttgatcaagcacttctgtttccccggactgagtatcaataggctgctcgcgcggctgaaggagaaaacgttcgttacccgaccaactacttcgagaagcttagtaccaccatgaacgaggcagggtgtttcgctcagcacaaccccagtgtagatcaggctgatgagtcactgcaacccccatgggcgaccatggcagtggctgcgttggcggcctgcccatggagaaatccatgggacgctctaattctgacatggtgtgaagtgcctattgagctaactggtagtcctccggcccctgattgcggctaatcctaactgcggagcacatgctcacaaaccagtgggtggtgtgtcgtaacgggcaactctgcagcggaaccgactactttgggtgtccgtgtttccttttattcctatattggctgcttatggtgacaatcaaaaagttgttaccatatagctattggattggccatccggtgtgcaacagggcaactgtttacctatttattggttttgtaccattatcactgaagtctgtgatcactctcaaattcattttgaccctcaacacaatcaaacgccaccatgggatggagctgtatcatcctcttcttggtagcaacagctaccggtgtgcactccgacatcgtgatgacccagactccactctccctgcccgtcacccctggagagcccgccagcattagctgcaggtctagcaagagcctcttgcacagcaatggcatcacttatttgtattggtacctgcaaaagccagggcagtctccacagctcctgatttatcaaatgtccaaccttgtctctggcgtccctgatcggttctccggttccgggtcaggcactgatttcacactgaaaatcagcagggtggaggctgaggatgttggagtttattactgcgctcagaatctagaacttccttacaccttcggcggagggaccaaggtggagatcaaatccagcgctagcaccaagggcccctccgtgttccccctggcccccagcagcaagagcaccagcggcggcacagccgctctgggctgcctggtcaaggactacttccccgagcccgtgaccgtgtcctggaacagcggagccctgacctccggcgtgcacaccttccccgccgtgctgcagagttctggcctgtatagcctgagcagcgtggtcaccgtgccttctagcagcctgggcacccagacctacatctgcaacgtgaaccacaagcccagcaacaccaaggtggacaagaaggtggagcccaagagctgcggagggggcggatccttctgggtgctggtggtggtgggcggcgtgctggcctgctacagcctgctggtgaccgtggccttcatcatcttctgggtgaggagcaagaggagcaggctgctgcacagcgactacatgaacatgacccccaggaggcccggccccaccaggaagcactaccagccctacgccccccccagggacttcgccgcctacaggagcagggtgaagttcagcaggagcgccgacgcccccgcctaccagcagggccagaaccagctgtataacgagctgaacctgggcaggagggaggagtacgacgtgctggacaagaggaggggcagggaccccgagatgggcggcaagcccaggaggaagaacccccaggagggcctgtataacgagctgcagaaggacaagatggccgaggcctacagcgagatcggcatgaagggcgagaggaggaggggcaagggccacgacggcctgtaccagggcctgagcaccgccaccaaggacacctacgacgccctgcacatgcaggccctgccccccaggtccggagagggcagaggaagtcttctaacatgcggtgacgtggaggagaatcccggccctagggtgagcaagggcgaggagctgttcaccggggtggtgcccatcctggtcgagctggacggcgacgtaaacggccacaagttcagcgtgtccggcgagggcgagggcgatgccacctacggcaagctgaccctgaagttcatctgcaccaccggcaagctgcccgtgccctggcccaccctcgtgaccaccctgacctacggcgtgcagtgcttcagccgctaccccgaccacatgaagcagcacgacttcttcaagtccgccatgcccgaaggctacgtccaggagcgcaccatcttcttcaaggacgacggcaactacaagacccgcgccgaggtgaagttcgagggcgacaccctggtgaaccgcatcgagctgaagggcatcgacttcaaggaggacggcaacatcctggggcacaagctggagtacaactacaacagccacaacgtctatatcatggccgacaagcagaagaacggcatcaaggtgaacttcaagatccgccacaacatcgaggacggcagcgtgcagctcgccgaccactaccagcagaacacccccatcggcgacggccccgtgctgctgcccgacaaccactacctgagcacccagtccgccctgagcaaagaccccaacgagaagcgcgatcacatggtcctgctggagttcgtgaccgccgccgggatcactctcggcatggacgagctgtacaagtga

SEQ ID NO: 50 - protein, 404 aa, Artificial sequence
  Anti-CD20-(GA101)-Fab VL-CL light chain-CD28ATD-CD28CSD-CD3zSSD fusion
DIVMTQTPLSLPVTPGEPASISCRSSKSLLHSNGITYLYWYLQKPGQSPQLLIYQMSNLVSGVPDRFSGSGSGTDFTLKISRVEAEDVGVYYCAQNLELPYTFGGGTKVEIKRTVAAPSVFIFPPSDEQLKSGTASVVCLLNNFYPREAKVQWKVDNALQSGNSQESVTEQDSKDSTYSLSSTLTLSKADYEKHKVYACEVTHQGLSSPVTKSFNRGECGGGGSFWVLVVVGGVLACYSLLVTVAFIIFWVRSKRSRLLHSDYMNMTPRRPGPTRKHYQPYAPPRDFAAYRSRVKFSRSADAPAYQQGQNQLYNELNLGRREEYDVLDKRRGRDPEMGGKPRRKNPQEGLYNELQKDKMAEAYSEIGMKGERRRGKGHDGLYQGLSTATKDTYDALHMQALPPR

SEQ ID NO: 51 - protein, 658 aa, Artificial sequence
  Anti-CD20-(GA101)-scFab-CD28ATD-CD28CSD-CD3zSSD fusion pETR17101
DIVMTQTPLSLPVTPGEPASISCRSSKSLLHSNGITYLYWYLQKPGQSPQLLIYQMSNLVSGVPDRFSGSGSGTDFTLKISRVEAEDVGVYYCAQNLELPYTFGGGTKVEIKRTVAAPSVFIFPPSDEQLKSGTASVVCLLNNFYPREAKVQWKVDNALQSGNSQESVTEQDSKDSTYSLSSTLTLSKADYEKHKVYACEVTHQGLSSPVTKSFNRGECGGGGSGGGGSGGGGSGGGGSGGGGSGGGGSGGQVQLVQSGAEVKKPGSSVKVSCKASGYAFSYSWINWVRQAPGQGLEWMGRIFPGDGDTDYNGKFKGRVTITADKSTSTAYMELSSLRSEDTAVYYCARNVFDGYWLVYWGQGTLVTVSSASTKGPSVFPLAPSSKSTSGGTAALGCLVKDYFPEPVTVSWNSGALTSGVHTFPAVLQSSGLYSLSSVVTVPSSSLGTQTYICNVNHKPSNTKVDKKVEPKSCGGGGSFWVLVVVGGVLACYSLLVTVAFIIFWVRSKRSRLLHSDYMNMTPRRPGPTRKHYQPYAPPRDFAAYRSRVKFSRSADAPAYQQGQNQLYNELNLGRREEYDVLDKRRGRDPEMGGKPRRKNPQEGLYNELQKDKMAEAYSEIGMKGERRRGKGHDGLYQGLSTATKDTYDALHMQALPPR

SEQ ID NO: 52 - protein, 473 aa, Artificial sequence
  Anti-CD20-(GA101)-scFab
DIVMTQTPLSLPVTPGEPASISCRSSKSLLHSNGITYLYWYLQKPGQSPQLLIYQMSNLVSGVPDRFSGSGSGTDFTLKISRVEAEDVGVYYCAQNLELPYTFGGGTKVEIKRTVAAPSVFIFPPSDEQLKSGTASVVCLLNNFYPREAKVQWKVDNALQSGNSQESVTEQDSKDSTYSLSSTLTLSKADYEKHKVYACEVTHQGLSSPVTKSFNRGECGGGGSGGGGSGGGGSGGGGSGGGGSGGGGSGGQVQLVQSGAEVKKPGSSVKVSCKASGYAFSYSWINWVRQAPGQGLEWMGRIFPGDGDTDYNGKFKGRVTITADKSTSTAYMELSSLRSEDTAVYYCARNVFDGYWLVYWGQGTLVTVSSASTKGPSVFPLAPSSKSTSGGTAALGCLVKDYFPEPVTVSWNSGALTSGVHTFPAVLQSSGLYSLSSVVTVPSSSLGTQTYICNVNHKPSNTKVDKKVEPKSC

SEQ ID NO: 53 - protein, 106 aa, Artificial sequence
  scFab-CL
RTVAAPSVFIFPPSDEQLKSGTASVVCLLNNFYPREAKVQWKVDNALQSGNSQESVTEQDSKDSTYSLSSTLTLSKADYEKHKVYACEVTHQGLSSPVTKSFNRGE

SEQ ID NO: 54 - protein, 32 aa, Artificial sequence
  (G4S)6G2 linker
GGGGSGGGGSGGGGSGGGGSGGGGSGGGGSGG

SEQ ID NO: 55 - DNA, 2031 bp, Artificial sequence
  Anti-CD20-(GA101)-scFab-CD28ATD-CD28CSD-CD3zSSD fusion pETR170101
atgggatggagctgtatcatcctcttcttggtagcaacagctacgggtgtgcattccgacatcgtgatgacccagactccactctccctgcccgtcacccctggagagcccgccagcattagctgcaggtctagcaagagcctcttgcacagcaatggcatcacttatttgtattggtacctgcaaaagccagggcagtctccacagctcctgatttatcaaatgtccaaccttgtctctggcgtccctgatcggttctccggttccgggtcaggcactgatttcacactgaaaatcagcagggtggaggctgaggatgttggagtttattactgcgctcagaatctagaacttccttacaccttcggcggagggaccaaggtggagatcaaacgtacggtggctgcaccatctgtcttcatcttcccgccatctgatgagcagttgaaatctggaactgcctctgttgtgtgcctgctgaataacttctatcccagagaggccaaagtacagtggaaggtggataacgccctccaatcgggtaactcccaggagagtgtcacagagcaggacagcaaggacagcacctacagcctcagcagcaccctgacgctgagcaaagcagactacgagaaacacaaagtctacgcctgcgaagtcacccatcagggcctgagctcgcccgtcacaaagagcttcaacaggggagagtgtggcggcggaggatctggtggcggaggtagtggtggtggtggatctggcggaggcggctccggcggaggtggaagcggaggtggtggttccggaggacaggtgcaattggtgcagtctggcgctgaagttaagaagcctgggagttcagtgaaggtctcctgcaaggcttcgggatacgccttcagctattcttggatcaattgggtgcggcaggcgcctggacaagggctcgagtggatgggacggatctttcccggcgatggggatactgactacaatgggaaattcaagggcagagtcacaattaccgccgacaaatccactagcacagcctatatggagctgagcagcctgagatctgaggacacggccgtgtattactgtgcaagaaatgtctttgatggttactggcttgtttactggggccagggaaccctggtcaccgtctcctcagctagcaccaagggcccctccgtgttccccctggcccccagcagcaagagcaccagcggcggcacagccgctctgggctgcctggtcaaggactacttccccgagcccgtgaccgtgtcctggaacagcggagccctgacctccggcgtgcacaccttccccgccgtgctgcagagttctggcctgtatagcctgagcagcgtggtcaccgtgccttctagcagcctgggcacccagacctacatctgcaacgtgaaccacaagcccagcaacaccaaggtggacaagaaggtggagcccaagagctgcggagggggcggatccttctgggtgctggtggtggtgggcggcgtgctggcctgctacagcctgctggtgaccgtggccttcatcatcttctgggtgaggagcaagaggagcaggctgctgcacagcgactacatgaacatgacccccaggaggcccggccccaccaggaagcactaccagccctacgccccccccagggacttcgccgcctacaggagcagggtgaagttcagcaggagcgccgacgcccccgcctaccagcagggccagaaccagctgtataacgagctgaacctgggcaggagggaggagtacgacgtgctggacaagaggaggggcagggaccccgagatgggcggcaagcccaggaggaagaacccccaggagggcctgtataacgagctgcagaaggacaagatggccgaggcctacagcgagatcggcatgaagggcgagaggaggaggggcaagggccacgacggcctgtaccagggcctgagcaccgccaccaaggacacctacgacgccctgcacatgcaggccctgccccccagg

SEQ ID NO: 56 - DNA, 336 bp, Artificial sequence
  scFab-VL
gacatcgtgatgacccagactccactctccctgcccgtcacccctggagagcccgccagcattagctgcaggtctagcaagagcctcttgcacagcaatggcatcacttatttgtattggtacctgcaaaagccagggcagtctccacagctcctgatttatcaaatgtccaaccttgtctctggcgtccctgatcggttctccggttccgggtcaggcactgatttcacactgaaaatcagcagggtggaggctgaggatgttggagtttattactgcgctcagaatctagaacttccttacaccttcggcggagggaccaaggtggagatcaaa

SEQ ID NO: 57 - DNA, 321 bp, Artificial sequence
  scFab-CL
cgtacggtggctgcaccatctgtcttcatcttcccgccatctgatgagcagttgaaatctggaactgcctctgttgtgtgcctgctgaataacttctatcccagagaggccaaagtacagtggaaggtggataacgccctccaatcgggtaactcccaggagagtgtcacagagcaggacagcaaggacagcacctacagcctcagcagcaccctgacgctgagcaaagcagactacgagaaacacaaagtctacgcctgcgaagtcacccatcagggcctgagctcgcccgtcacaaagagcttcaacaggggagagtgt

SEQ ID NO: 58 - DNA, 357 bp, Artificial sequence
  Anti-CD20-(GA101)- scFab-VH
caggtgcaattggtgcagtctggcgctgaagttaagaagcctgggagttcagtgaaggtctcctgcaaggcttcgggatacgccttcagctattcttggatcaattgggtgcggcaggcgcctggacaagggctcgagtggatgggacggatctttcccggcgatggggatactgactacaatgggaaattcaagggcagagtcacaattaccgccgacaaatccactagcacagcctatatggagctgagcagcctgagatctgaggacacggccgtgtattactgtgcaagaaatgtctttgatggttactggcttgtttactggggccagggaaccctggtcaccgtctcctca

SEQ ID NO: 59 - DNA, 2806 bp, Artificial sequence
  Anti-CD20-(GA101)-scFab-CD28ATD-CD28CSD-CD3zSSD-eGFP fusion pETR170101
atggagctgtatcatcctcttcttggtagcaacagctacgggtgtgcattccgacatcgtgatgacccagactccactctccctgcccgtcacccctggagagcccgccagcattagctgcaggtctagcaagagcctcttgcacagcaatggcatcacttatttgtattggtacctgcaaaagccagggcagtctccacagctcctgatttatcaaatgtccaaccttgtctctggcgtccctgatcggttctccggttccgggtcaggcactgatttcacactgaaaatcagcagggtggaggctgaggatgttggagtttattactgcgctcagaatctagaacttccttacaccttcggcggagggaccaaggtggagatcaaacgtacggtggctgcaccatctgtcttcatcttcccgccatctgatgagcagttgaaatctggaactgcctctgttgtgtgcctgctgaataacttctatcccagagaggccaaagtacagtggaaggtggataacgccctccaatcgggtaactcccaggagagtgtcacagagcaggacagcaaggacagcacctacagcctcagcagcaccctgacgctgagcaaagcagactacgagaaacacaaagtctacgcctgcgaagtcacccatcagggcctgagctcgcccgtcacaaagagcttcaacaggggagagtgtggcggcggaggatctggtggcggaggtagtggtggtggtggatctggcggaggcggctccggcggaggtggaagcggaggtggtggttccggaggacaggtgcaattggtgcagtctggcgctgaagttaagaagcctgggagttcagtgaaggtctcctgcaaggcttcgggatacgccttcagctattcttggatcaattgggtgcggcaggcgcctggacaagggctcgagtggatgggacggatctttcccggcgatggggatactgactacaatgggaaattcaagggcagagtcacaattaccgccgacaaatccactagcacagcctatatggagctgagcagcctgagatctgaggacacggccgtgtattactgtgcaagaaatgtctttgatggttactggcttgtttactggggccagggaaccctggtcaccgtctcctcagctagcaccaagggcccctccgtgttccccctggcccccagcagcaagagcaccagcggcggcacagccgctctgggctgcctggtcaaggactacttccccgagcccgtgaccgtgtcctggaacagcggagccctgacctccggcgtgcacaccttccccgccgtgctgcagagttctggcctgtatagcctgagcagcgtggtcaccgtgccttctagcagcctgggcacccagacctacatctgcaacgtgaaccacaagcccagcaacaccaaggtggacaagaaggtggagcccaagagctgcggagggggcggatccttctgggtgctggtggtggtgggcggcgtgctggcctgctacagcctgctggtgaccgtggccttcatcatcttctgggtgaggagcaagaggagcaggctgctgcacagcgactacatgaacatgacccccaggaggcccggccccaccaggaagcactaccagccctacgccccccccagggacttcgccgcctacaggagcagggtgaagttcagcaggagcgccgacgcccccgcctaccagcagggccagaaccagctgtataacgagctgaacctgggcaggagggaggagtacgacgtgctggacaagaggaggggcagggaccccgagatgggcggcaagcccaggaggaagaacccccaggagggcctgtataacgagctgcagaaggacaagatggccgaggcctacagcgagatcggcatgaagggcgagaggaggaggggcaagggccacgacggcctgtaccagggcctgagcaccgccaccaaggacacctacgacgccctgcacatgcaggccctgccccccaggtccggagagggcagaggaagtcttctaacatgcggtgacgtggaggagaatcccggccctagggtgagcaagggcgaggagctgttcaccggggtggtgcccatcctggtcgagctggacggcgacgtaaacggccacaagttcagcgtgtccggcgagggcgagggcgatgccacctacggcaagctgaccctgaagttcatctgcaccaccggcaagctgcccgtgccctggcccaccctcgtgaccaccctgacctacggcgtgcagtgcttcagccgctaccccgaccacatgaagcagcacgacttcttcaagtccgccatgcccgaaggctacgtccaggagcgcaccatcttcttcaaggacgacggcaactacaagacccgcgccgaggtgaagttcgagggcgacaccctggtgaaccgcatcgagctgaagggcatcgacttcaaggaggacggcaacatcctggggcacaagctggagtacaactacaacagccacaacgtctatatcatggccgacaagcagaagaacggcatcaaggtgaacttcaagatccgccacaacatcgaggacggcagcgtgcagctcgccgaccactaccagcagaacacccccatcggcgacggccccgtgctgctgcccgacaaccactacctgagcacccagtccgccctgagcaaagaccccaacgagaagcgcgatcacatggtcctgctggagttcgtgaccgccgccgggatcactctcggcatggacgagctgtacaagtga

SEQ ID NO: 60 - protein, 436 aa, Artificial sequence
  Anti-CD20-(GA101)-ds-scFv-CD28ATD-CD28CSD-CD3zSSD fusion pETR17162
QVQLVQSGAEVKKPGSSVKVSCKASGYAFSYSWINWVRQAPGQCLEWMGRIFPGDGDTDYNGKFKGRVTITADKSTSTAYMELSSLRSEDTAVYYCARNVFDGYWLVYWGQGTLVTVSSGGGGSGGGGSGGGGSGGGGSDIVMTQTPLSLPVTPGEPASISCRSSKSLLHSNGITYLYWYLQKPGQSPQLLIYQMSNLVSGVPDRFSGSGSGTDFTLKISRVEAEDVGVYYCAQNLELPYTFGCGTKVEIKGGGGSFWVLVVVGGVLACYSLLVTVAFIIFWVRSKRSRLLHSDYMNMTPRRPGPTRKHYQPYAPPRDFAAYRSRVKFSRSADAPAYQQGQNQLYNELNLGRREEYDVLDKRRGRDPEMGGKPRRKNPQEGLYNELQKDKMAEAYSEIGMKGERRRGKGHDGLYQGLSTATKDTYDALHMQALPPR

SEQ ID NO: 61 - protein, 251 aa, Artificial sequence
  Anti-CD20-(GA101)-ds-scFv
QVQLVQSGAEVKKPGSSVKVSCKASGYAFSYSWINWVRQAPGQCLEWMGRIFPGDGDTDYNGKFKGRVTITADKSTSTAYMELSSLRSEDTAVYYCARNVFDGYWLVYWGQGTLVTVSSGGGGSGGGGSGGGGSGGGGSDIVMTQTPLSLPVTPGEPASISCRSSKSLLHSNGITYLYWYLQKPGQSPQLLIYQMSNLVSGVPDRFSGSGSGTDFTLKISRVEAEDVGVYYCAQNLELPYTFGCGTKVEIK

SEQ ID NO: 62 - protein, 119 aa, Artificial sequence
  Anti-CD20-(GA101)- ds-Fab VH
QVQLVQSGAEVKKPGSSVKVSCKASGYAFSYSWINWVRQAPGQCLEWMGRIFPGDGDTDYNGKFKGRVTITADKSTSTAYMELSSLRSEDTAVYYCARNVFDGYWLVYWGQGTLVTVSS

SEQ ID NO: 63 - protein, 112 aa, Artificial sequence
  Anti-CD20-(GA101)- ds-Fab VL
DIVMTQTPLSLPVTPGEPASISCRSSKSLLHSNGITYLYWYLQKPGQSPQLLIYQMSNLVSGVPDRFSGSGSGTDFTLKISRVEAEDVGVYYCAQNLELPYTFGCGTKVEIK

SEQ ID NO: 64 - DNA, 1364 bp, Artificial sequence
  Anti-CD20-(GA101)-ds-Fab-CD28ATD-CD28CSD-CD3zSSD fusion pETR17162
atgggatggagctgtatcatcctcttcttggtagcaacagctaccggtgtgcattcccaggtgcaattggtgcagtctggcgctgaagttaagaagcctgggagttcagtgaaggtctcctgcaaggcttccggttacgccttcagctattcttggatcaattgggtgcggcaggcgcctggacaatgtctcgagtggatgggacggatctttcccggcgatggggatactgactacaatgggaaattcaagggcagagtcacaattaccgccgacaaatccactagcacagcctatatggagctgagcagcctgagatctgaggacacggccgtgtattactgtgcaagaaatgtctttgatggttactggcttgtttactggggccagggaaccctggtcaccgtctcctcaggagggggcggaagtggtggcgggggaagcggcgggggtggcagcggagggggcggatctgacatcgtgatgacccagactccactctccctgcccgtcacccctggagagcccgccagcattagctgcaggtctagcaagagcctcttgcacagcaatggcatcacttatttgtattggtacctgcaaaagccagggcagtctccacagctcctgatttatcaaatgtccaaccttgtctctggcgtccctgaccgcttctccggttccgggtcaggcactgatttcacactgaaaatcagcagggtggaggctgaggatgttggagtttattactgcgctcagaatctagaacttccttacaccttcggctgtgggaccaaggtggagatcaaggagggggcggatccttctgggtgctggtggtggtgggcggcgtgctggcctgctacagcctgctggtgaccgtggccttcatcatcttctgggtgaggagcaagaggagcaggctgctgcacagcgactacatgaacatgacccccaggaggcccggccccaccaggaagcactaccagccctacgccccccccagggacttcgccgcctacaggagcagggtgaagttcagcaggagcgccgacgcccccgcctaccagcagggccagaaccagctgtataacgagctgaacctgggcaggagggaggagtacgacgtgctggacaagaggaggggcagggaccccgagatgggcggcaagcccaggaggaagaacccccaggagggcctgtataacgagctgcagaaggacaagatggccgaggcctacagcgagatcggcatgaagggcgagaggaggaggggcaagggccacgacggcctgtaccagggcctgagcaccgccaccaaggacacctacgacgccctgcacatgcaggccctgccccccagg

SEQ ID NO: 65 - DNA, 357 bp, Artificial sequence
  Anti-CD20-(GA101)- ds-Fab VH
caggtgcaattggtgcagtctggcgctgaagttaagaagcctgggagttcagtgaaggtctcctgcaaggcttccggttacgccttcagctattcttggatcaattgggtgcggcaggcgcctggacaatgtctcgagtggatgggacggatctttcccggcgatggggatactgactacaatgggaaattcaagggcagagtcacaattaccgccgacaaatccactagcacagcctatatggagctgagcagcctgagatctgaggacacggccgtgtattactgtgcaagaaatgtctttgatggttactggcttgtttactggggccagggaaccctggtcaccgtctcctca

SEQ ID NO: 66 - DNA, 336 bp, Artificial sequence
  Anti-CD20-(GA101)- ds-Fab VL
gacatcgtgatgacccagactccactctccctgcccgtcacccctggagagcccgccagcattagctgcaggtctagcaagagcctcttgcacagcaatggcatcacttatttgtattggtacctgcaaaagccagggcagtctccacagctcctgatttatcaaatgtccaaccttgtctctggcgtccctgaccgcttctccggttccgggtcaggcactgatttcacactgaaaatcagcagggtggaggctgaggatgttggagtttattactgcgctcagaatctagaacttccttacaccttcggctgtgggaccaaggtggagatcaaa

SEQ ID NO: 67 - DNA, 2151 bp, Artificial sequence
  Anti-CD20-(GA101)-ds-scFv-CD28ATD-CD28CSD-CD3zSSD-eGFP fusion pETR17162
gccaccatgggatggagctgtatcatcctcttcttggtagcaacagctaccggtgtgcattcccaggtgcaattggtgcagtctggcgctgaagttaagaagcctgggagttcagtgaaggtctcctgcaaggcttccggttacgccttcagctattcttggatcaattgggtgcggcaggcgcctggacaatgtctcgagtggatgggacggatctttcccggcgatggggatactgactacaatgggaaattcaagggcagagtcacaattaccgccgacaaatccactagcacagcctatatggagctgagcagcctgagatctgaggacacggccgtgtattactgtgcaagaaatgtctttgatggttactggcttgtttactggggccagggaaccctggtcaccgtctcctcaggagggggcggaagtggtggcgggggaagcggcgggggtggcagcggagggggcggatctgacatcgtgatgacccagactccactctccctgcccgtcacccctggagagcccgccagcattagctgcaggtctagcaagagcctcttgcacagcaatggcatcacttatttgtattggtacctgcaaaagccagggcagtctccacagctcctgatttatcaaatgtccaaccttgtctctggcgtccctgaccgcttctccggttccgggtcaggcactgatttcacactgaaaatcagcagggtggaggctgaggatgttggagtttattactgcgctcagaatctagaacttccttacaccttcggctgtgggaccaaggtggagatcaaaggagggggcggatccttctgggtgctggtggtggtgggcggcgtgctggcctgctacagcctgctggtgaccgtggccttcatcatcttctgggtgaggagcaagaggagcaggctgctgcacagcgactacatgaacatgacccccaggaggcccggccccaccaggaagcactaccagccctacgccccccccagggacttcgccgcctacaggagcagggtgaagttcagcaggagcgccgacgcccccgcctaccagcagggccagaaccagctgtataacgagctgaacctgggcaggagggaggagtacgacgtgctggacaagaggaggggcagggaccccgagatgggcggcaagcccaggaggaagaacccccaggagggcctgtataacgagctgcagaaggacaagatggccgaggcctacagcgagatcggcatgaagggcgagaggaggaggggcaagggccacgacggcctgtaccagggcctgagcaccgccaccaaggacacctacgacgccctgcacatgcaggccctgccccccaggtccggagagggcagaggaagtcttctaacatgcggtgacgtggaggagaatcccggccctagggtgagcaagggcgaggagctgttcaccggggtggtgcccatcctggtcgagctggacggcgacgtaaacggccacaagttcagcgtgtccggcgagggcgagggcgatgccacctacggcaagctgaccctgaagttcatctgcaccaccggcaagctgcccgtgccctggcccaccctcgtgaccaccctgacctacggcgtgcagtgcttcagccgctaccccgaccacatgaagcagcacgacttcttcaagtccgccatgcccgaaggctacgtccaggagcgcaccatcttcttcaaggacgacggcaactacaagacccgcgccgaggtgaagttcgagggcgacaccctggtgaaccgcatcgagctgaagggcatcgacttcaaggaggacggcaacatcctggggcacaagctggagtacaactacaacagccacaacgtctatatcatggccgacaagcagaagaacggcatcaaggtgaacttcaagatccgccacaacatcgaggacggcagcgtgcagctcgccgaccactaccagcagaacacccccatcggcgacggccccgtgctgctgcccgacaaccactacctgagcacccagtccgccctgagcaaagaccccaacgagaagcgcgatcacatggtcctgctggagttcgtgaccgccgccgggatcactctcggcatggacgagctgtacaagtga

SEQ ID NO: 68 - protein, 164 aa, Homo sapiens
MKWKALFTAAILQAQLPITEAQSFGLLDPKLCYLLDGILFIYGVILTALFLRVKFSRSADAPAYQQGQNQLYNELNLGRREEYDVLDKRRGRDPEMGGKPQRRKNPQEGLYNELQKDKMAEAYSEIGMKGERRRGKGHDGLYQGLSTATKDTYDALHMQALPPR

SEQ ID NO: 69 - DNA, 492 bp, Homo sapiens
atgaagtggaaggcgcttttcaccgcggccatcctgcaggcacagttgccgattacagaggcacagagctttggcctgctggatcccaaactctgctacctgctggatggaatcctcttcatctatggtgtcattctcactgccttgttcctgagagtgaagttcagcaggagcgcagagccccccgcgtaccagcagggccagaaccagctctataacgagctcaatctaggacgaagagaggagtacgatgttttggacaagagacgtggccgggaccctgagatggggggaaagccgagaaggaagaaccctcaggaaggcctgtacaatgaactgcagaaagataagatggcggaggcctacagtgagattgggatgaaaggcgagcgccggaggggcaaggggcacgatggcctttaccagggtctcagtacagccaccaaggacacctacgacgcccttcacatgcaggccctgccccctcgctaa

SEQ ID NO: 70 - protein, 164 aa, Mus musculus
MKWKVSVLACILHVRFPGAEAQSFGLLDPKLCYLLDGILFIYGVIITALYLRAKFSRSAETAANLQDPNQLYNELNLGRREEYDVLEKKRARDPEMGGKQQRRRNPQEGVYNALQKDKMAEAYSEIGTKGERRRGKGHDGLYQGLSTATKDTYDALHMQTLAPR

SEQ ID NO: 71 - DNA, 495 bp, Mus musculus
atgaagtggaaagtgtctgttctcgcctgcatcctccacgtgcggttcccaggagcagaggcacagagctttggtctgctggatcccaaactctgctacttgctagatggaatcctcttcatctacggagtcatcatcacagccctgtacctgagagcaaaattcagcaggagtgcagagactgctgccaacctgcaggaccccaaccagctctacaatgagctcaatctagggcgaagagaggaatatgacgtcttggagaagaagcgggctcgggatccagagatgggaggcaaacagcagaggaggaggaacccccaggaaggcgtatacaatgcactgcagaaagacaagatggcagaagcctacagtgagatcggcacaaaaggcgagaggcggagaggcaaggggcacgatggcctttaccagggtctcagcactgccaccaaggacacctatgatgccctgcatatgcagaccctggcccctcgctaa

SEQ ID NO: 72 - DNA, 660 bp, Homo sapiens
atgctgcgcctgctgctggcgctgaacctgtttccgagcattcaggtgaccggcaacaaaattctggtgaaacagagcccgatgctggtggcgtatgataacgcggtgaacctgagctgcaaatatagctataacctgtttagccgcgaatttcgcgcgagcctgcataaaggcctggatagcgcggtggaagtgtgcgtggtgtatggcaactatagccagcagctgcaggtgtatagcaaaaccggctttaactgcgatggcaaactgggcaacgaaagcgtgaccttttatctgcagaacctgtatgtgaaccagaccgatatttatttttgcaaaattgaagtgatgtatccgccgccgtatctggataacgaaaaaagcaacggcaccattattcatgtgaaaggcaaacatctgtgcccgagcccgctgtttccgggcccgagcaaaccgttttgggtgctggtggtggtgggcggcgtgctggcgtgctatagcctgctggtgaccgtggcgtttattattttttgggtgcgcagcaaacgcagccgcctgctgcatagcgattatatgaacatgaccccgcgccgcccgggcccgacccgcaaacattatcagccgtatgcgccgccgcgcgattttgcggcgtatcgcagc

SEQ ID NO: 73 - protein, 220 aa, Homo sapiens
MLRLLLALNLFPSIQVTGNKILVKQSPMLVAYDNAVNLSCKYSYNLFSREFRASLHKGLDSAVEVCVVYGNYSQQLQVYSKTGFNCDGKLGNESVTFYLQNLYVNQTDIYFCKIEVMYPPPYLDNEKSNGTIIHVKGKHLCPSPLFPGPSKPFWVLVVVGGVLACYSLLVTVAFIIFWVRSKRSRLLHSDYMNMTPRRPGPTRKHYQPYAPPRDFAAYRS

SEQ ID NO: 74 - DNA, 654 bp, Mus musculus
atgaccctgcgcctgctgtttctggcgctgaacttttttagcgtgcaggtgaccgaaaacaaaattctggtgaaacagagcccgctgctggtggtggatagcaacgaagtgagcctgagctgccgctatagctataacctgctggcgaaagaatttcgcgcgagcctgtataaaggcgtgaacagcgatgtggaagtgtgcgtgggcaacggcaactttacctatcagccgcagtttcgcagcaacgcggaatttaactgcgatggcgattttgataacgaaaccgtgacctttcgcctgtggaacctgcatgtgaaccataccgatatttatttttgcaaaattgaatttatgtatccgccgccgtatctggataacgaacgcagcaacggcaccattattcatattaaagaaaaacatctgtgccatacccagagcagcccgaaactgttttgggcgctggtggtggtggcgggcgtgctgttttgctatggcctgctggtgaccgtggcgctgtgcgtgatttggaccaacagccgccgcaaccgcctgctgcagagcgattatatgaacatgaccccgcgccgcccgggcctgacccgcaaaccgtatcagccgtatgcgccggcgcgcgattttgcggcgtatcgcccg

SEQ ID NO: 75 - protein, 218 aa, Mus musculus
MTLRLLFLALNFFSVQVTENKILVKQSPLLVVDSNEVSLSCRYSYNLLAKEFRASLYKGVNSDVEVCVGNGNFTYQPQFRSNAEFNCDGDFDNETVTFRLWNLHVNHTDIYFCKIEFMYPPPYLDNERSNGTIIHIKEKHLCHTQSSPKLFWALVVVAGVLFCYGLLVTVALCVIWTNSRRNRLLQSDYMNMTPRRPGLTRKPYQPYAPARDFAAYRP

SEQ ID NO: 76 - protein, 4 aa, Artificial sequence
  CD28 YMNM
YMNM

SEQ ID NO: 77 - protein, 4 aa, Artificial sequence
  CD28 PYAP
PYAP

SEQ ID NO: 78 - protein, 21 aa, Artificial sequence
  Signal peptide
ATMGWSCIILFLVATATGVHS

SEQ ID NO: 79 - DNA, 57 bp, Artificial sequence
  Signal peptide DNA sequence
atgggatggagctgtatcatcctcttcttggtagcaacagctaccggtgtgcactcc

SEQ ID NO: 80 - protein, 116 aa, Artificial sequence
  Anti-WT1 (33F05) VH
QVQLQESGPGLVKPSETLSLTCTVSGGSINSYYWSWIRQPPGKGLEWIGYIYYSGSTNYNPSLKSRVTISVDTSKNQFSLKLSSVTAADTAVYYCARSYYEAFDYWGQGTLVTVSS

SEQ ID NO: 81 - protein, 107 aa, Artificial sequence
  Anti-WT1 (33F05) VL
SSELTQDPAVSVALGQTVRITCQGDSLRSYYASWYQQKPGQAPVLVIYGKNNRPSGIPDRFSGSSSGNTASLTITGAQAEDEADYYCNSPDMNGNAVFGGGTKLTVL

SEQ ID NO: 82 - protein, 120 aa, Artificial sequence
  Anti-WT1 (11D06) VH
QVQLVQSGAEVKKPGSSVKVSCKASGGTFSSYAISWVRQAPGQGLEWMGGIIPIFGTANYAQKFQGRVTITADKSTSTAYMELSSLRSEDTAVYYCARSIELWWGGFDYWGQGTTVTVSS

SEQ ID NO: 83 - protein, 106 aa, Artificial sequence
  Anti-WT1 (11D06) VL
DIQMTQSPSTLSASVGDRVTITCRASQSISSWLAWYQQKPGKAPKLLIYDASSLESGVPSRFSGSGSGTEFTLTIGSLQPDDFATYYCQQYEDYTTFGQGTKVEIK

SEQ ID NO: 84 - protein, 119 aa, Artificial sequence
  Anti-WT1 (33H09) VH
QVQLVQSGAEVKKPGSSVKVSCKASGGTFSSYAISWVRQAPGQGLEWMGGIIPIFGTANYAQKFQGRVTITADKSTSTAYMELSSLRSEDTAVYYCARGSYDLFSLDYWGQGTTVTVSS

SEQ ID NO: 85 - protein, 106 aa, Artificial sequence
  Anti-WT1 (33H09) VL
DIQMTQSPSTLSASVGDRVTITCRASQSISSWLAWYQQKPGKAPKLLIYDASSLESGVPSRFSGSGSGTEFTLTISSLQPDDFATYYCQQYYDGITFGQGTKVEIK

SEQ ID NO: 86 - protein, 119 aa, Artificial sequence
  Anti-WT1 (5E11) VH
QVQLVQSGAEVKKPGSSVKVSCKASGGTFSSYAISWVRQAPGQGLEWMGGIIPIFGTANYAQKFQGRVTITADKSTSTAYMELSSLRSEDTAVYYCARSSYDLYSFDYWGQGTTVTVSS

SEQ ID NO: 87 - protein, 108 aa, Artificial sequence
  Anti-WT1 (5E11) VL
DIQMTQSPSTLSASVGDRVTITCRASQSISSWLAWYQQKPGKAPKLLIYDASSLESGVPSRFSGSGSGTEFTLTISSLQPDDFATYYCQQYSFPPMITFGQGTKVEIK

SEQ ID NO: 88 - protein, 5 aa, Artificial sequence
  Anti-CD3 HCDR1 Kabat
TYAMN

SEQ ID NO: 89 - protein, 19 aa, Artificial sequence
  Anti-CD3 HCDR2 Kabat
RIRSKYNNYATYYADSVKG

SEQ ID NO: 90 - protein, 14 aa, Artificial sequence
  Anti-CD3 HCDR3 Kabat
HGNFGNSYVSWFAY

SEQ ID NO: 91 - protein, 14 aa, Artificial sequence
  Anti-CD3 LCDR1 Kabat
GSSTGAVTTSNYAN

SEQ ID NO: 92 - protein, 7 aa, Artificial sequence
  Anti-CD3 LCDR2 Kabat
GTNKRAP

SEQ ID NO: 93 - protein, 9 aa, Artificial sequence
  Anti-CD3 LCDR3 Kabat
ALWYSNLWV